European Patent Application EP 4 382 598 A1, published June 12, 2024. Title: Method for preserving or transporting stem cells in non-frozen state. Applicant: RAINBOW INC. Application JP, filed August 1, 2022. The sequence listing filed with the application follows.

SEQUENCE LISTING (9 sequences)

SEQ ID NO: 1 - protein, 571 aa, synthetic construct
  REGION 1..571: note = Amino acid sequence of recombinant collagen-like peptide (RCP)
GAPGAPGLQGAPGLQGMPGERGAAGLPGPKGERGDAGPKGADGAPGAPGLQGMPGERGAAGLPGPKGERGDAGPKGADGAPGKDGVRGLAGPIGPPGERGAAGLPGPKGERGDAGPKGADGAPGKDGVRGLAGPIGPPGPAGAPGAPGLQGMPGERGAAGLPGPKGERGDAGPKGADGAPGKDGVRGLAGPPGAPGLQGAPGLQGMPGERGAAGLPGPKGERGDAGPKGADGAPGAPGLQGMPGERGAAGLPGPKGERGDAGPKGADGAPGKDGVRGLAGPIGPPGERGAAGLPGPKGERGDAGPKGADGAPGKDGVRGLAGPIGPPGPAGAPGAPGLQGMPGERGAAGLPGPKGERGDAGPKGADGAPGKDGVRGLAGPPGAPGLQGAPGLQGMPGERGAAGLPGPKGERGDAGPKGADGAPGAPGLQGMPGERGAAGLPGPKGERGDAGPKGADGAPGKDGVRGLAGPIGPPGERGAAGLPGPKGERGDAGPKGADGAPGKDGVRGLAGPIGPPGPAGAPGAPGLQGMPGERGAAGLPGPKGERGDAGPKGADGAPGKDGVRGLAGPPG

SEQ ID NO: 2 - protein, 4 aa, synthetic construct
  REGION 1..4: note = Amino acid sequence of cell adhesion signal sequence
REDV

SEQ ID NO: 3 - protein, 5 aa, synthetic construct
  REGION 1..5: note = Amino acid sequence of cell adhesion signal sequence
YIGSR

SEQ ID NO: 4 - protein, 5 aa, synthetic construct
  REGION 1..5: note = Amino acid sequence of cell adhesion signal sequence
PDSGR

SEQ ID NO: 5 - protein, 7 aa, synthetic construct
  REGION 1..7: note = Amino acid sequence of cell adhesion signal sequence
RYVVLPR

SEQ ID NO: 6 - protein, 6 aa, synthetic construct
  REGION 1..6: note = Amino acid sequence of cell adhesion signal sequence
LGTIPG

SEQ ID NO: 7 - protein, 10 aa, synthetic construct
  REGION 1..10: note = Amino acid sequence of cell adhesion signal sequence
RNIAEIIKDI

SEQ ID NO: 8 - protein, 5 aa, synthetic construct
  REGION 1..5: note = Amino acid sequence of cell adhesion signal sequence
IKVAV

SEQ ID NO: 9 - protein, 4 aa, synthetic construct
  REGION 1..4: note = Amino acid sequence of cell adhesion signal sequence
DGEA